European Patent Specification EP 3 760 734 B1, published August 20, 2025. Title: Nucleic acid modification and identification method. Applicant: IMBA - INSTITUT FÜR MOLEKULARE BIOTECHNOLOGIE GMBH. The sequence listing filed with the application follows.

SEQUENCE LISTING (11 sequences)

SEQ ID NO: 1 - RNA, 76 nt, Artificial Sequence
  5L-let-7-3L
acacucuuucccuacacgacgcucuuccgaucuugagguaguagguuguauaguagaucggaagagcacacgucuc

SEQ ID NO: 2 - RNA, 76 nt, Artificial Sequence; identical to SEQ ID NO: 1
  5L-let-7-s4U-p9-3L
  modified_base (42)..(42): s4u

SEQ ID NO: 3 - RNA, 21 nt, Artificial Sequence
  let-7-s6G sequence
  modified_base (8)..(8): s6g
ugagguaguagguuguauagu

SEQ ID NO: 4 - DNA, 34 bp, Artificial Sequence
  RT primer
gtgactggagttcagacgtgtgctcttccgatct

SEQ ID NO: 5 - DNA, 58 bp, Artificial Sequence
  Solexa_PCR_fwd
aatgatacggcgaccaccgagatctacactctttccctacacgacgctcttccgatct

SEQ ID NO: 6 - DNA, 64 bp, Artificial Sequence
  Solexa_IDX_rev
  misc_feature (25)..(30): n is a, c, g, or t
caagcagaagacggcatacgagatnnnnnngtgactggagttcagacgtgtgctcttccgatct

SEQ ID NO: 7 - DNA, 21 bp, Artificial Sequence
  mature dme-let-7 sequence
tgaggtagtaggttgtatagt

SEQ ID NO: 8 - RNA, 77 nt, Artificial Sequence
  synthetic RNA oligonucleotide
  misc_structure (44)..(44): 5-Br-U
acacucuuucccuacacgacgcucuuccgaucuugagguaguuagguuguauaguagaucggaagagcacacgucuc

SEQ ID NO: 9 - DNA, 34 bp, Artificial Sequence; identical to SEQ ID NO: 4
  primer

SEQ ID NO: 10 - DNA, 58 bp, Artificial Sequence; identical to SEQ ID NO: 5
  primer

SEQ ID NO: 11 - DNA, 64 bp, Artificial Sequence; identical to SEQ ID NO: 6
  primer
  misc_feature (25)..(30): n is a, c, g, or t